European Patent Application EP 4 494 762 A1, published January 22, 2025. Title: Methods and devices for processing microparticles. Applicant: BLINK AG. Application EP. The sequence listing filed with the application follows.

SEQUENCE LISTING (3 sequences)

SEQ ID NO: 1 - DNA, 20 bp, synthetic construct
  source 1..20: mol_type = other DNA
gcatcgatgaagaacgcagc

SEQ ID NO: 2 - DNA, 19 bp, synthetic construct
  source 1..19: mol_type = other DNA
gacgctcaaacaggcatgc

SEQ ID NO: 3 - DNA, 25 bp, synthetic construct
  source 1..25: mol_type = other DNA
  misc_binding 1: bound_moiety = ATTO647N
  misc_binding 25: bound_moiety = BHQ2
cgtgaatcatcgagtctttgaacgc